European Patent Specification EP 4 006 046 B1, published March 19, 2025. Title: Novel steviol glycoside and production method for same, and sweetener composition containing same. Applicant: SUNTORY HOLDINGS LIMITED. The sequence listing filed with the application follows.

SEQUENCE LISTING (72 sequences)

SEQ ID NO: 1 - DNA, 635 bp, Stevia rebaudiana
atcaacctgagcaacaaagttactgacaacacgaccatcgtcaatgcacatcctaggaccataagtattgaatatcctcgcaatcctcacctgcaggttttttttttttttttttaatcaaaccaaattaatgattctttctgtagataaccagagattatatattatcctaaaatttaaacaaaactactctctacgtccccaaaataccatgtgccattgattacaatcaaataaacttaatcttattagtaaactgatggaaaacaaaatttagataaataaagccttggacttcttatgccaaatttatttttattttttttcaccaactttaattaatattgaccataaacattcttgtttgtatgactcaactttaattcttttttctttcattttgataacatcttttaaacaggactcactatttgaacattatgttccattttcttttaaaaaaaaataatgtggaaataataactgattaacataataataattttgagaaagataatatatagaaacaaatttactttacaataataagcttatcttgatttatggcatgcaatataattttaattgccctttaacctttaatatagtttgtgtaacagtcaacttgttttggt

SEQ ID NO: 2 - DNA, 635 bp, Stevia rebaudiana
atcaacctgagcaacaaagttactgacaacacgaccatcgtcaatgcacatcctaggaccataagtattgaatatcctcgcaatcctcacctgcaggttttttttttttttttttaatcaaaccaaattaatgattctttctgtagataaccagagattatatattatcctaaaatttaaacaaaactactctctacgtccccaaaataccatgtgccattgattacaatcaaataaacttaatcttattagtaaactgatggaaaacaaaatttagataaataaagccttggactttttatgccaaatttatttttattttttttccccaactttaattaatattgaccataaacatttttgtttgtatgactcaactttaatttttttttttttcattttgataacattttttaaacaggactccctatttgaacattatgttccatttttttttaaaaaaaaataatgtggaaataataactgattaacataataataattttgagaaagataatatatagaaacaaatttactttacaataataagcttatcttgatttatggcatgcaatataattttaattgccctttaacctttaatatagtttgtgtaacagtcaacttgttttggt

SEQ ID NO: 3 - DNA, 21 bp, Stevia rebaudiana
ccttggacttcttatgccaaa

SEQ ID NO: 4 - DNA, 21 bp, Stevia rebaudiana
ccttggactttttatgccaaa

SEQ ID NO: 5 - DNA, 41 bp, Stevia rebaudiana
ataaataaagccttggacttcttatgccaaatttattttta

SEQ ID NO: 6 - DNA, 41 bp, Stevia rebaudiana
ataaataaagccttggactttttatgccaaatttattttta

SEQ ID NO: 7 - DNA, 51 bp, Stevia rebaudiana
tttagataaataaagccttggacttcttatgccaaatttatttttattttt

SEQ ID NO: 8 - DNA, 51 bp, Stevia rebaudiana
tttagataaataaagccttggactttttatgccaaatttatttttattttt

SEQ ID NO: 9 - DNA, 21 bp, Stevia rebaudiana
attttttttcaccaactttaa

SEQ ID NO: 10 - DNA, 21 bp, Stevia rebaudiana
attttttttccccaactttaa

SEQ ID NO: 11 - DNA, 41 bp, Stevia rebaudiana
atttatttttattttttttcaccaactttaattaatattga

SEQ ID NO: 12 - DNA, 41 bp, Stevia rebaudiana
atttatttttattttttttccccaactttaattaatattga

SEQ ID NO: 13 - DNA, 51 bp, Stevia rebaudiana
gccaaatttatttttattttttttcaccaactttaattaatattgaccata

SEQ ID NO: 14 - DNA, 51 bp, Stevia rebaudiana
gccaaatttatttttattttttttccccaactttaattaatattgaccata

SEQ ID NO: 15 - DNA, 21 bp, Stevia rebaudiana
cataaacattcttgtttgtat

SEQ ID NO: 16 - DNA, 21 bp, Stevia rebaudiana
cataaacatttttgtttgtat

SEQ ID NO: 17 - DNA, 41 bp, Stevia rebaudiana
taatattgaccataaacattcttgtttgtatgactcaactt

SEQ ID NO: 18 - DNA, 41 bp, Stevia rebaudiana
taatattgaccataaacatttttgtttgtatgactcaactt

SEQ ID NO: 19 - DNA, 51 bp, Stevia rebaudiana
ttaattaatattgaccataaacattcttgtttgtatgactcaactttaatt

SEQ ID NO: 20 - DNA, 51 bp, Stevia rebaudiana
ttaattaatattgaccataaacatttttgtttgtatgactcaactttaatt

SEQ ID NO: 21 - DNA, 21 bp, Stevia rebaudiana
aactttaattcttttttcttt

SEQ ID NO: 22 - DNA, 21 bp, Stevia rebaudiana
aactttaattttttttttttt

SEQ ID NO: 23 - DNA, 41 bp, Stevia rebaudiana
tgtatgactcaactttaattcttttttctttcattttgata

SEQ ID NO: 24 - DNA, 41 bp, Stevia rebaudiana
tgtatgactcaactttaatttttttttttttcattttgata

SEQ ID NO: 25 - DNA, 50 bp, Stevia rebaudiana
ttgtttgtatgactcaactttaattcttttttctttcattttgataacat

SEQ ID NO: 26 - DNA, 50 bp, Stevia rebaudiana
ttgtttgtatgactcaactttaatttttttttttttcattttgataacat

SEQ ID NO: 27 - DNA, 21 bp, Stevia rebaudiana
attcttttttctttcattttg

SEQ ID NO: 28 - DNA, 21 bp, Stevia rebaudiana
atttttttttttttcattttg

SEQ ID NO: 29 - DNA, 35 bp, Stevia rebaudiana
aactttaattcttttttctttcattttgataacat

SEQ ID NO: 30 - DNA, 35 bp, Stevia rebaudiana
aactttaatttttttttttttcattttgataacat

SEQ ID NO: 31 - DNA, 45 bp, Stevia rebaudiana
gactcaactttaattcttttttctttcattttgataacatctttt

SEQ ID NO: 32 - DNA, 45 bp, Stevia rebaudiana
gactcaactttaatttttttttttttcattttgataacatttttt

SEQ ID NO: 33 - DNA, 21 bp, Stevia rebaudiana
ttgataacatcttttaaacag

SEQ ID NO: 34 - DNA, 21 bp, Stevia rebaudiana
ttgataacattttttaaacag

SEQ ID NO: 35 - DNA, 35 bp, Stevia rebaudiana
tttcattttgataacatcttttaaacaggactcac

SEQ ID NO: 36 - DNA, 35 bp, Stevia rebaudiana
tttcattttgataacattttttaaacaggactccc

SEQ ID NO: 37 - DNA, 45 bp, Stevia rebaudiana
ttttctttcattttgataacatcttttaaacaggactcactattt

SEQ ID NO: 38 - DNA, 45 bp, Stevia rebaudiana
ttttttttcattttgataacattttttaaacaggactccctattt

SEQ ID NO: 39 - DNA, 21 bp, Stevia rebaudiana
aacaggactcactatttgaac

SEQ ID NO: 40 - DNA, 21 bp, Stevia rebaudiana
aacaggactccctatttgaac

SEQ ID NO: 41 - DNA, 35 bp, Stevia rebaudiana
tcttttaaacaggactcactatttgaacattatgt

SEQ ID NO: 42 - DNA, 35 bp, Stevia rebaudiana
ttttttaaacaggactccctatttgaacattatgt

SEQ ID NO: 43 - DNA, 45 bp, Stevia rebaudiana
taacatcttttaaacaggactcactatttgaacattatgttccat

SEQ ID NO: 44 - DNA, 45 bp, Stevia rebaudiana
taacattttttaaacaggactccctatttgaacattatgttccat

SEQ ID NO: 45 - DNA, 21 bp, Stevia rebaudiana
gttccattttcttttaaaaaa

SEQ ID NO: 46 - DNA, 21 bp, Stevia rebaudiana
gttccatttttttttaaaaaa

SEQ ID NO: 47 - DNA, 35 bp, Stevia rebaudiana
acattatgttccattttcttttaaaaaaaaataat

SEQ ID NO: 48 - DNA, 35 bp, Stevia rebaudiana
acattatgttccatttttttttaaaaaaaaataat

SEQ ID NO: 49 - DNA, 45 bp, Stevia rebaudiana
tttgaacattatgttccattttcttttaaaaaaaaataatgtgga

SEQ ID NO: 50 - DNA, 45 bp, Stevia rebaudiana
tttgaacattatgttccatttttttttaaaaaaaaataatgtgga

SEQ ID NO: 51 - DNA, 25 bp, Artificial Sequence
  Synthetic DNA
atcaacctgagcaacaaagttactg

SEQ ID NO: 52 - DNA, 25 bp, Artificial Sequence
  Synthetic DNA
accaaaacaagttgactgttacaca

SEQ ID NO: 53 - protein, 306 aa, Stevia rebaudiana
MGSELTYRHQDTLPGASESYSPKPNKQSVTRVVRYILREQRLVFVLLGIAIATSVFTLLPSSTNTVTDAYSVSESVQLMNPQRSVYPARFNMGGKIPLGLKRKGLRIVVTGGAGFVGSHLVDRLIARGDSVIVVDNFFTGNKDNVMHHFGNPRFELIRHDVVEPLLLEVDQIYHLACPASPVHYKFNPTNVVGTLNMLGLAKRVGARFLLTSTSEVYGDPLQHPQVETYWGNVNPIAQVVQETIDPNASIEFKPNTEDDPHKRKPDITKAKELLGWKPKVPLRKGLPMMVSDFRRRIFGDQNNPSA

SEQ ID NO: 54 - DNA, 921 bp, Stevia rebaudiana
atgggatctgagttaacataccggcaccaagataccctaccgggggcgtcggaatcttactcgccgaagcctaacaagcagtccgtgactcgcgtcgttcgttacatcctccgtgagcagcgtctcgtatttgtgcttttgggcattgcaatcgctacctccgtcttcacgctcctcccatcatccacaaacaccgtcaccgatgcctattccgtctctgaatcggtccagttgatgaacccgcagcgatccgtgtatcctgcgagattcaatatgggcgggaagattccgctaggtttgaaacgaaaggggttaaggattgtggtgaccggtggtgcaggttttgtcggaagtcatctagttgaccggttgattgcgaggggagacagtgtgattgttgttgataatttcttcactggtaacaaggataacgtgatgcatcactttggaaaccctagatttgagcttattcgtcacgacgttgttgagcctttgctactcgaggtcgatcagatctatcacctggcttgtcctgcttcccctgttcattacaaattcaacccgacaaatgtggtagggacattgaacatgttagggttggcgaagagggttggtgcgcggttcttgctaacaagcaccagcgaggtatacggtgatcctttacagcatcctcaagtcgaaacctactggggcaacgtcaatcctatcgcccaggtggtccaggaaacgatagacccaaacgcaagcatagagttcaaaccaaacacagaagacgacccacacaaacggaagccggatatcacaaaggctaaggaactcctgggttggaagcccaaggtccctcttcgcaaaggtctccccatgatggtttctgacttcaggcgccgcatttttggtgaccaaaacaacccatccgcttaa

SEQ ID NO: 55 - DNA, 24 bp, Artificial Sequence
  Synthetic DNA
cctgttcattacaaattcaacccg

SEQ ID NO: 56 - DNA, 25 bp, Artificial Sequence
  Synthetic DNA
aaccctaacatgttcaatgtcccta

SEQ ID NO: 57 - DNA, 316 bp, Stevia rebaudiana
cgggcgtgttgtgagtaattttatagctcaagcacttcggttagtcctccattataatcagaatcagtatttttaattttaaatatatttggttaatcttaattcttgcagcgatgaacctttaaccgttcaagcccctggaacccaaacccgcagtttctgttacgtctctgatatggtattttgaaaaataatatgattatacatttatgatataactggtgacgcgtgtcaaacattgacttttttttaaaccgtataggttgatgggcttgttaaactaatggaaggtgaaaacactggaccaatcaacatc

SEQ ID NO: 58 - DNA, 331 bp, Stevia rebaudiana
cgggcgtgttgtgagtaattttatagctcaagcacttcggttagtcctccattataatcagaatcagtatttttaattttaaatatattttttttaaatatatttggttaatcttaattcttgcagcgatgaacctttaaccgttcaagcccctggaacccaaacccgcagtttctgttacgtctctgatatggtattttgaaaaataatatgattatacatttatgatataactggtgacgcgtgtcaaacattgacttttttttaaaccgtataggttgatgggcttgttaaactaatggaaggtgaaaacactggaccaatcaacatc

SEQ ID NO: 59 - DNA, 183 bp, Stevia rebaudiana
aacccaattggtaagcgtgcatctctgtttattttttgttaattattgtgtatttgttgaattatcaattatattggtgattctttcttctttaaaataaataaaaaccgtgaaattatggtttttattatttatgtattttgcaggagttaggagttgctatgatgaaggaaaacgcgtggc

SEQ ID NO: 60 - DNA, 183 bp, Stevia rebaudiana
aacccaattggtaagcgtgcatctctgtttattttttgttaattattgtgtatttgttgaattatcaattatattggtgattctttcttctttaaaaaaaaaaaaaaccggggaaataagggttttattatttatgtattttgcaggagttaggagttgctatgatgaaggaaaacgcgtggc

SEQ ID NO: 61 - protein, 251 aa, Stevia rebaudiana
MANNASNGEHKSSKPPPTPSPLRNSKFFQSNMRILVTGGAGFIGSHLVDKLMENEKNEVIVADNYFTGSKDNLRKWIGHPRFELIRHDVTEPLLVEVDQIYHLACPASPIFYKHNPVKTIAETLMFDYHRQHGIEIRIARIFNTYGPRMNIDDGRVVDGLVKLMEGENTGPINIGNPGEFTMIELAEMVKELINPKIEIKMVENTPDDPRQRKPDITNAKKMLGWEPKIKLRDGLPLMEADFRLRLGVAKK

SEQ ID NO: 62 - DNA, 936 bp, Stevia rebaudiana
atggcgaataatgcttcaaacggagaacataaatcttcaaaaccgcctccaacgccttctcctttaaggaactccaaattctttcagtcaaacatgaggatattggttactggtggtgctggatttatcggctctcacttggtggataaacttatggaaaatgaaaagaatgaggtaattgttgctgataattactttactggctcaaaagataatcttagaaaatggattggtcatccaagatttgagcttattcgtcatgatgtcactgaaccattgctagttgaggttgatcagatttatcatcttgcatgccccgcttcaccaattttttataaacacaatcctgtaaagacgattaagacgaatgtaattggcacactaaatatgcttggtcttgcgaagcgagtcggggcaaggattttgcttacctcaacatctgaggtatacggtgatcctcttgtgcatccgcaaccagagagttactggggtaatgtcaacccgattggagttcggagttgctatgatgaaggaaaacgtgtggcagagactctgatgtttgattatcacaggcaacatggaatagaaataagaattgcgcgtattttcaacacatatggaccccggatgaatattgatgacgggcgtgttgttgatgggcttgttaaactaatggaaggtgaaaacactggaccaatcaacatcggtaatccaggtgaattcacaatgatcgaactcgctgagatggttaaggagcttattaatccgaaaatagagattaagatggtggaaaacacacccgatgatccacgacaaagaaaacccgacatcacaaatgcgaagaagatgcttggatgggagccgaagatcaaactgcgcgatggacttccgctcatggaagctgattttaggctgaggcttggagttgccaagaag

SEQ ID NO: 63 - protein, 313 aa, Stevia rebaudiana
MANNASNGEHKVTKPPPTPSPLRNSKFLQSNMRILVTGGAGFIGSHLVDKLMENEKNEVIVADNYFTGSKDNLRKWIGHPRFELIRHDVTEKLLVEVDQIYHLACPASPIFYKYNPVKTIKTNVIGTLNMLGLAKRVGARILLTSTSEVYGDPLVHPQPETYWGNVNPIGVRSCYDEGKRVAETLMFDYHRQHGIEIRIARIFNTYGPRMNIDDGRVVDGLIRLMEGENTGPINIGNPGEFTMIELAETVKELINPKIEIKMVENTPDDPRQRKPDITNAKKMLGWEPKIKLRDGLPLMEADFRLRLGVAKKI

SEQ ID NO: 64 - DNA, 942 bp, Stevia rebaudiana
atggcaaataacgcttcaaatggtgaacataaagttacaaaaccacctccaaccccatctcctctgcgtaattctaaattcttgcagtcaaatatgaggatattggttactggtggtgctggatttatcggatctcacctagtggataaactgatggaaaatgaaaagaatgaggtgattgttgctgataattattttactggttcaaaagacaaccttagaaagtggattggtcatccaagatttgagcttattcgacatgatgtcacagaaaagttgctggttgaagttgatcagatataccatcttgcatgtcctgcttcacccattttttataaatacaatcctgttaaaacgataaagactaatgttattggcacactaaatatgcttggtcttgccaagcgagttggagcaaggattttgcttacctcgacctcggaggtatatggtgatcctctcgtgcatccacaacctgagacctactggggtaatgtcaacccaattggagttaggagttgctatgatgaaggaaaacgcgtggcagagactttgatgtttgattatcacagacaacatggcatagaaataagaattgctcgtattttcaacacatatggaccccggatgaacatcgatgacggacgtgtcgttgatgggcttattcggctgatggaaggtgagaacaccggaccaatcaacattggtaatccgggtgaatttacaatgattgaactcgctgaaacagtcaaagagcttataaatccaaaaatagagattaagatggtggaaaacacgcctgatgatccaagacaaagaaaaccggatattacaaatgctaaaaagatgcttggatgggagcctaagattaaattgcgcgatggtcttccgcttatggaagcagactttaggttaaggcttggagttgcaaagaagatataa

SEQ ID NO: 65 - DNA, 25 bp, Artificial Sequence
  Synthetic DNA
atcagatttatcatcttgcatgccc

SEQ ID NO: 66 - DNA, 25 bp, Artificial Sequence
  Synthetic DNA
tgccaattacattcgtcttaatcgt

SEQ ID NO: 67 - DNA, 25 bp, Artificial Sequence
  Synthetic DNA
aaaagttgctggttgaagttgatca

SEQ ID NO: 68 - DNA, 24 bp, Artificial Sequence
  Synthetic DNA
cacactaaatatgcttggtcttgc

SEQ ID NO: 69 - DNA, 24 bp, Artificial Sequence
  Synthetic DNA
cgccatcctccgtcttgatcttgc

SEQ ID NO: 70 - DNA, 20 bp, Artificial Sequence
  Synthetic DNA
ccgttcggcggtggtggtaa

SEQ ID NO: 71 - DNA, 25 bp, Artificial Sequence
  Synthetic DNA
tcactcttgaagtggagagttccga

SEQ ID NO: 72 - DNA, 20 bp, Artificial Sequence
  Synthetic DNA
gcctctgttggtccggtggg